European Patent Application EP 4 349 852 A1, published April 10, 2024. Title: RECOMBINANT ADENO-ASSOCIATED VIRUS HAVING VARIANT CAPSID, AND APPLICATION THEREOF. Applicant: JIANGSU HENGRUI PHARMACEUTICALS CO., LTD. SHANGHAI SHENGDI PHARMACEUTICAL CO., LTD. The sequence listing filed with the application follows.

SEQUENCE LISTING (41 sequences)

SEQ ID NO: 1 - protein, 735 aa, AAV2 [sequence omitted]

SEQ ID NO: 2 - protein, 745 aa, AAV2.7m8
MAADGYLPDWLEDTLSEGIRQWWKLKPGPPPPKPAERHKDDSRGLVLPGYKYLGPFNGLDKGEPVNEADAAALEHDKAYDRQLDSGDNPYLKYNHADAEFQERLKEDTSFGGNLGRAVFQAKKRVLEPLGLVEEPVKTAPGKKRPVEHSPVEPDSSSGTGKAGQQPARKRLNFGQTGDADSVPDPQPLGQPPAAPSGLGTNTMATGSGAPMADNNEGADGVGNSSGNWHCDSTWMGDRVITTSTRTWALPTYNNHLYKQISSQSGASNDNHYFGYSTPWGYFDFNRFHCHFSPRDWQRLINNNWGFRPKRLNFKLFNIQVKEVTQNDGTTTIANNLTSTVQVFTDSEYQLPYVLGSAHQGCLPPFPADVFMVPQYGYLTLNNGSQAVGRSSFYCLEYFPSQMLRTGNNFTFSYTFEDVPFHSSYAHSQSLDRLMNPLIDQYLYYLSRTNTPSGTTTQSRLQFSQAGASDIRDQSRNWLPGPCYRQQRVSKTSADNNNSEYSWTGATKYHLNGRDSLVNPGPAMASHKDDEEKFFPQSGVLIFGKQGSEKTNVDIEKVMITDEEEIRTTNPVATEQYGSVSTNLQRGNLALGETTRPARQAATADVNTQGVLPGMVWQDRDVYLQGPIWAKIPHTDGHFHPSPLMGGFGLKHPPPQILIKNTPVPANPSTTFSAAKFASFITQYSTGQVSVEIEWELQKENSKRWNPEIQYTSNYNKSINVDFTVDTNGVYSEPRPIGTRYLTRNL

SEQ ID NO: 3 - protein, 745 aa, Artificial Sequence
  AAV2 seq1
MAADGYLPDWLEDTLSEGIRQWWKLKPGPPPPKPAERHKDDSRGLVLPGYKYLGPFNGLDKGEPVNEADAAALEHDKAYDRQLDSGDNPYLKYNHADAEFQERLKEDTSFGGNLGRAVFQAKKRVLEPLGLVEEPVKTAPGKKRPVEHSPVEPDSSSGTGKAGQQPARKRLNFGQTGDADSVPDPQPLGQPPAAPSGLGTNTMATGSGAPMADNNEGADGVGNSSGNWHCDSTWMGDRVITTSTRTWALPTYNNHLYKQISSQSGASNDNHYFGYSTPWGYFDFNRFHCHFSPRDWQRLINNNWGFRPKRLNFKLFNIQVKEVTQNDGTTTIANNLTSTVQVFTDSEYQLPYVLGSAHQGCLPPFPADVFMVPQYGYLTLNNGSQAVGRSSFYCLEYFPSQMLRTGNNFTFSYTFEDVPFHSSYAHSQSLDRLMNPLIDQYLYYLSRTNTPSGTTTQSRLQFSQAGASDIRDQSRNWLPGPCYRQQRVSKTSADNNNSEYSWTGATKYHLNGRDSLVNPGPAMASHKDDEEKFFPQSGVLIFGKQGSEKTNVDIEKVMITDEEEIRTTNPVATEQYGSVSTNLQRGNLALAETTRPARQAATADVNTQGVLPGMVWQDRDVYLQGPIWAKIPHTDGHFHPSPLMGGFGLKHPPPQILIKNTPVPANPSTTFSAAKFASFITQYSTGQVSVEIEWELQKENSKRWNPEIQYTSNYNKSINVDFTVDTNGVYSEPRPIGTRYLTRNL

SEQ ID NO: 4 - protein, 745 aa, Artificial Sequence
  AAV2 seq2
MAADGYLPDWLEDTLSEGIRQWWKLKPGPPPPKPAERHKDDSRGLVLPGYKYLGPFNGLDKGEPVNEADAAALEHDKAYDRQLDSGDNPYLKYNHADAEFQERLKEDTSFGGNLGRAVFQAKKRVLEPLGLVEEPVKTAPGKKRPVEHSPVEPDSSSGTGKAGQQPARKRLNFGQTGDADSVPDPQPLGQPPAAPSGLGTNTMATGSGAPMADNNEGADGVGNSSGNWHCDSTWMGDRVITTSTRTWALPTYNNHLYKQISSQSGASNDNHYFGYSTPWGYFDFNRFHCHFSPRDWQRLINNNWGFRPKRLNFKLFNIQVKEVTQNDGTTTIANNLTSTVQVFTDSEYQLPYVLGSAHQGCLPPFPADVFMVPQYGYLTLNNGSQAVGRSSFYCLEYFPSQMLRTGNNFTFSYTFEDVPFHSSYAHSQSLDRLMNPLIDQYLYYLSRTNTPSGTTTQSRLQFSQAGASDIRDQSRNWLPGPCYRQQRVSKTSADNNNSEYSWTGATKYHLNGRDSLVNPGPAMASHKDDEEKFFPQSGVLIFGKQGSEKTNVDIEKVMITDEEEIRTTNPVATEQYGSVSTNLQRGNLALGDTTRPARQAATADVNTQGVLPGMVWQDRDVYLQGPIWAKIPHTDGHFHPSPLMGGFGLKHPPPQILIKNTPVPANPSTTFSAAKFASFITQYSTGQVSVEIEWELQKENSKRWNPEIQYTSNYNKSINVDFTVDTNGVYSEPRPIGTRYLTRNL

SEQ ID NO: 5 - protein, 745 aa, Artificial Sequence
  AAV2 seq3
MAADGYLPDWLEDTLSEGIRQWWKLKPGPPPPKPAERHKDDSRGLVLPGYKYLGPFNGLDKGEPVNEADAAALEHDKAYDRQLDSGDNPYLKYNHADAEFQERLKEDTSFGGNLGRAVFQAKKRVLEPLGLVEEPVKTAPGKKRPVEHSPVEPDSSSGTGKAGQQPARKRLNFGQTGDADSVPDPQPLGQPPAAPSGLGTNTMATGSGAPMADNNEGADGVGNSSGNWHCDSTWMGDRVITTSTRTWALPTYNNHLYKQISSQSGASNDNHYFGYSTPWGYFDFNRFHCHFSPRDWQRLINNNWGFRPKRLNFKLFNIQVKEVTQNDGTTTIANNLTSTVQVFTDSEYQLPYVLGSAHQGCLPPFPADVFMVPQYGYLTLNNGSQAVGRSSFYCLEYFPSQMLRTGNNFTFSYTFEDVPFHSSYAHSQSLDRLMNPLIDQYLYYLSRTNTPSGTTTQSRLQFSQAGASDIRDQSRNWLPGPCYRQQRVSKTSADNNNSEYSWTGATKYHLNGRDSLVNPGPAMASHKDDEEKFFPQSGVLIFGKQGSEKTNVDIEKVMITDEEEIRTTNPVATEQYGSVSTNLQRGNLALGETTRNARQAATADVNTQGVLPGMVWQDRDVYLQGPIWAKIPHTDGHFHPSPLMGGFGLKHPPPQILIKNTPVPANPSTTFSAAKFASFITQYSTGQVSVEIEWELQKENSKRWNPEIQYTSNYNKSINVDFTVDTNGVYSEPRPIGTRYLTRNL

SEQ ID NO: 6 - protein, 745 aa, Artificial Sequence
  AAV2 seq4
MAADGYLPDWLEDTLSEGIRQWWKLKPGPPPPKPAERHKDDSRGLVLPGYKYLGPFNGLDKGEPVNEADAAALEHDKAYDRQLDSGDNPYLKYNHADAEFQERLKEDTSFGGNLGRAVFQAKKRVLEPLGLVEEPVKTAPGKKRPVEHSPVEPDSSSGTGKAGQQPARKRLNFGQTGDADSVPDPQPLGQPPAAPSGLGTNTMATGSGAPMADNNEGADGVGNSSGNWHCDSTWMGDRVITTSTRTWALPTYNNHLYKQISSQSGASNDNHYFGYSTPWGYFDFNRFHCHFSPRDWQRLINNNWGFRPKRLNFKLFNIQVKEVTQNDGTTTIANNLTSTVQVFTDSEYQLPYVLGSAHQGCLPPFPADVFMVPQYGYLTLNNGSQAVGRSSFYCLEYFPSQMLRTGNNFTFSYTFEDVPFHSSYAHSQSLDRLMNPLIDQYLYYLSRTNTPSGTTTQSRLQFSQAGASDIRDQSRNWLPGPCYRQQRVSKTSADNNNSEYSWTGATKYHLNGRDSLVNPGPAMASHKDDEEKFFPQSGVLIFGKQGSEKTNVDIEKVMITDEEEIRTTNPVATEQYGSVSTNLQRGNLAKADTTKNARQAATADVNTQGVLPGMVWQDRDVYLQGPIWAKIPHTDGHFHPSPLMGGFGLKHPPPQILIKNTPVPANPSTTFSAAKFASFITQYSTGQVSVEIEWELQKENSKRWNPEIQYTSNYNKSINVDFTVDTNGVYSEPRPIGTRYLTRNL

SEQ ID NO: 7 - protein, 745 aa, Artificial Sequence
  AAV2 seq5
MAADGYLPDWLEDTLSEGIRQWWKLKPGPPPPKPAERHKDDSRGLVLPGYKYLGPFNGLDKGEPVNEADAAALEHDKAYDRQLDSGDNPYLKYNHADAEFQERLKEDTSFGGNLGRAVFQAKKRVLEPLGLVEEPVKTAPGKKRPVEHSPVEPDSSSGTGKAGQQPARKRLNFGQTGDADSVPDPQPLGQPPAAPSGLGTNTMATGSGAPMADNNEGADGVGNSSGNWHCDSTWMGDRVITTSTRTWALPTYNNHLYKQISSQSGASNDNHYFGYSTPWGYFDFNRFHCHFSPRDWQRLINNNWGFRPKRLNFKLFNIQVKEVTQNDGTTTIANNLTSTVQVFTDSEYQLPYVLGSAHQGCLPPFPADVFMVPQYGYLTLNNGSQAVGRSSFYCLEYFPSQMLRTGNNFTFSYTFEDVPFHSSYAHSQSLDRLMNPLIDQYLYYLSRTNTPSGTTTQSRLQFSQAGASDIRDQSRNWLPGPCYRQQRVSKTSADNNNSEYSWTGATKYHLNGRDSLVNPGPAMASHKDDEEKFFPQSGVLIFGKQGSEKTNVDIEKVMITDEEEIRTTNPVATEQYGSVSTNLQRGNLAKDDTTRNARQAATADVNTQGVLPGMVWQDRDVYLQGPIWAKIPHTDGHFHPSPLMGGFGLKHPPPQILIKNTPVPANPSTTFSAAKFASFITQYSTGQVSVEIEWELQKENSKRWNPEIQYTSNYNKSINVDFTVDTNGVYSEPRPIGTRYLTRNL

SEQ ID NO: 8 - protein, 745 aa, Artificial Sequence
  AAV2 seq6
MAADGYLPDWLEDTLSEGIRQWWKLKPGPPPPKPAERHKDDSRGLVLPGYKYLGPFNGLDKGEPVNEADAAALEHDKAYDRQLDSGDNPYLKYNHADAEFQERLKEDTSFGGNLGRAVFQAKKRVLEPLGLVEEPVKTAPGKKRPVEHSPVEPDSSSGTGKAGQQPARKRLNFGQTGDADSVPDPQPLGQPPAAPSGLGTNTMATGSGAPMADNNEGADGVGNSSGNWHCDSTWMGDRVITTSTRTWALPTYNNHLYKQISSQSGASNDNHYFGYSTPWGYFDFNRFHCHFSPRDWQRLINNNWGFRPKRLNFKLFNIQVKEVTQNDGTTTIANNLTSTVQVFTDSEYQLPYVLGSAHQGCLPPFPADVFMVPQYGYLTLNNGSQAVGRSSFYCLEYFPSQMLRTGNNFTFSYTFEDVPFHSSYAHSQSLDRLMNPLIDQYLYYLSRTNTPSGTTTQSRLQFSQAGASDIRDQSRNWLPGPCYRQQRVSKTSADNNNSEYSWTGATKYHLNGRDSLVNPGPAMASHKDDEEKFFPQSGVLIFGKQGSEKTNVDIEKVMITDEEEIRTTNPVATEQYGSVSTNLQRGNLALADTTKNARQAATADVNTQGVLPGMVWQDRDVYLQGPIWAKIPHTDGHFHPSPLMGGFGLKHPPPQILIKNTPVPANPSTTFSAAKFASFITQYSTGQVSVEIEWELQKENSKRWNPEIQYTSNYNKSINVDFTVDTNGVYSEPRPIGTRYLTRNL

SEQ ID NO: 9 - protein, 746 aa, Artificial Sequence
  AAV9 seq2
MAADGYLPDWLEDNLSEGIREWWALKPGAPQPKANQQHQDNARGLVLPGYKYLGPGNGLDKGEPVNAADAAALEHDKAYDQQLKAGDNPYLKYNHADAEFQERLKEDTSFGGNLGRAVFQAKKRLLEPLGLVEEAAKTAPGKKRPVEQSPQEPDSSAGIGKSGAQPAKKRLNFGQTGDTESVPDPQPIGEPPAAPSGVGSLTMASGGGAPVADNNEGADGVGSSSGNWHCDSQWLGDRVITTSTRTWALPTYNNHLYKQISNSTSGGSSNDNAYFGYSTPWGYFDFNRFHCHFSPRDWQRLINNNWGFRPKRLNFKLFNIQVKEVTDNNGVKTIANNLTSTVQVFTDSDYQLPYVLGSAHEGCLPPFPADVFMIPQYGYLTLNDGSQAVGRSSFYCLEYFPSQMLRTGNNFQFSYEFENVPFHSSYAHSQSLDRLMNPLIDQYLYYLSKTINGSGQNQQTLKFSVAGPSNMAVQGRNYIPGPSYRQQRVSTTVTQNNNSEFAWPGASSWALNGRNSLMNPGPAMASHKEGEDRFFPLSGSLIFGKQGTGRDNVDADKVMITNEEEIKTTNPVATESYGQVATNHQSAQLALGDTTRPAAQAQTGWVQNQGILPGMVWQDRDVYLQGPIWAKIPHTDGNFHPSPLMGGFGMKHPPPQILIKNTPVPADPPTAFNKDKLNSFITQYSTGQVSVEIEWELQKENSKRWNPEIQYTSNYYKSNNVEFAVNTEGVYSEPRPIGTRYLTRNL

SEQ ID NO: 10 - protein, 239 aa, Artificial Sequence
  Amino acid sequence of EGFP
MVSKGEELFTGVVPILVELDGDVNGHKFSVSGEGEGDATYGKLTLKFICTTGKLPVPWPTLVTTLTYGVQCFSRYPDHMKQHDFFKSAMPEGYVQERTIFFKDDGNYKTRAEVKFEGDTLVNRIELKGIDFKEDGNILGHKLEYNYNSHNVYIMADKQKNGIKVNFKIRHNIEDGSVQLADHYQQNTPIGDGPVLLPDNHYLSTQSALSKDPNEKRDHMVLLEFVTAAGITLGMDELYK

SEQ ID NO: 11 - protein, 7 aa, Artificial Sequence
  seq1 (without linker)
LAETTRP

SEQ ID NO: 12 - protein, 7 aa, Artificial Sequence
  seq2 (without linker)
LGDTTRP

SEQ ID NO: 13 - protein, 7 aa, Artificial Sequence
  seq3 (without linker)
LGETTRN

SEQ ID NO: 14 - protein, 7 aa, Artificial Sequence
  seq4 (without linker)
KADTTKN

SEQ ID NO: 15 - protein, 7 aa, Artificial Sequence
  seq5 (without linker)
KDDTTRN

SEQ ID NO: 16 - protein, 7 aa, Artificial Sequence
  seq6 (without linker)
LADTTKN

SEQ ID NO: 17 - protein, 10 aa, Artificial Sequence
  seq1
LALAETTRPA

SEQ ID NO: 18 - protein, 10 aa, Artificial Sequence
  seq2
LALGDTTRPA

SEQ ID NO: 19 - protein, 10 aa, Artificial Sequence
  seq3
LALGETTRNA

SEQ ID NO: 20 - protein, 10 aa, Artificial Sequence
  seq4
LAKADTTKNA

SEQ ID NO: 21 - protein, 10 aa, Artificial Sequence
  seq5
LAKDDTTRNA

SEQ ID NO: 22 - protein, 10 aa, Artificial Sequence
  seq6
LALADTTKNA

SEQ ID NO: 23 - protein, 745 aa, Artificial Sequence
  Amino acid sequence of AAV2 seq2 capsid (708V)
MAADGYLPDWLEDTLSEGIRQWWKLKPGPPPPKPAERHKDDSRGLVLPGYKYLGPFNGLDKGEPVNEADAAALEHDKAYDRQLDSGDNPYLKYNHADAEFQERLKEDTSFGGNLGRAVFQAKKRVLEPLGLVEEPVKTAPGKKRPVEHSPVEPDSSSGTGKAGQQPARKRLNFGQTGDADSVPDPQPLGQPPAAPSGLGTNTMATGSGAPMADNNEGADGVGNSSGNWHCDSTWMGDRVITTSTRTWALPTYNNHLYKQISSQSGASNDNHYFGYSTPWGYFDFNRFHCHFSPRDWQRLINNNWGFRPKRLNFKLFNIQVKEVTQNDGTTTIANNLTSTVQVFTDSEYQLPYVLGSAHQGCLPPFPADVFMVPQYGYLTLNNGSQAVGRSSFYCLEYFPSQMLRTGNNFTFSYTFEDVPFHSSYAHSQSLDRLMNPLIDQYLYYLSRTNTPSGTTTQSRLQFSQAGASDIRDQSRNWLPGPCYRQQRVSKTSADNNNSEYSWTGATKYHLNGRDSLVNPGPAMASHKDDEEKFFPQSGVLIFGKQGSEKTNVDIEKVMITDEEEIRTTNPVATEQYGSVSTNLQRGNLALGDTTRPARQAATADVNTQGVLPGMVWQDRDVYLQGPIWAKIPHTDGHFHPSPLMGGFGLKHPPPQILIKNTPVPANPSTTFSAAKFASFITQYSTGQVSVEIEWELQKENSKRWNPEIQYTSNYNKSVNVDFTVDTNGVYSEPRPIGTRYLTRNL

SEQ ID NO: 24 - protein, 745 aa, Artificial Sequence
  Amino acid sequence of AAV2 seq3 capsid (708V)
MAADGYLPDWLEDTLSEGIRQWWKLKPGPPPPKPAERHKDDSRGLVLPGYKYLGPFNGLDKGEPVNEADAAALEHDKAYDRQLDSGDNPYLKYNHADAEFQERLKEDTSFGGNLGRAVFQAKKRVLEPLGLVEEPVKTAPGKKRPVEHSPVEPDSSSGTGKAGQQPARKRLNFGQTGDADSVPDPQPLGQPPAAPSGLGTNTMATGSGAPMADNNEGADGVGNSSGNWHCDSTWMGDRVITTSTRTWALPTYNNHLYKQISSQSGASNDNHYFGYSTPWGYFDFNRFHCHFSPRDWQRLINNNWGFRPKRLNFKLFNIQVKEVTQNDGTTTIANNLTSTVQVFTDSEYQLPYVLGSAHQGCLPPFPADVFMVPQYGYLTLNNGSQAVGRSSFYCLEYFPSQMLRTGNNFTFSYTFEDVPFHSSYAHSQSLDRLMNPLIDQYLYYLSRTNTPSGTTTQSRLQFSQAGASDIRDQSRNWLPGPCYRQQRVSKTSADNNNSEYSWTGATKYHLNGRDSLVNPGPAMASHKDDEEKFFPQSGVLIFGKQGSEKTNVDIEKVMITDEEEIRTTNPVATEQYGSVSTNLQRGNLALGETTRNARQAATADVNTQGVLPGMVWQDRDVYLQGPIWAKIPHTDGHFHPSPLMGGFGLKHPPPQILIKNTPVPANPSTTFSAAKFASFITQYSTGQVSVEIEWELQKENSKRWNPEIQYTSNYNKSVNVDFTVDTNGVYSEPRPIGTRYLTRNL

SEQ ID NO: 25 - protein, 745 aa, Artificial Sequence
  Amino acid sequence of AAV2 seq4 capsid (708V)
MAADGYLPDWLEDTLSEGIRQWWKLKPGPPPPKPAERHKDDSRGLVLPGYKYLGPFNGLDKGEPVNEADAAALEHDKAYDRQLDSGDNPYLKYNHADAEFQERLKEDTSFGGNLGRAVFQAKKRVLEPLGLVEEPVKTAPGKKRPVEHSPVEPDSSSGTGKAGQQPARKRLNFGQTGDADSVPDPQPLGQPPAAPSGLGTNTMATGSGAPMADNNEGADGVGNSSGNWHCDSTWMGDRVITTSTRTWALPTYNNHLYKQISSQSGASNDNHYFGYSTPWGYFDFNRFHCHFSPRDWQRLINNNWGFRPKRLNFKLFNIQVKEVTQNDGTTTIANNLTSTVQVFTDSEYQLPYVLGSAHQGCLPPFPADVFMVPQYGYLTLNNGSQAVGRSSFYCLEYFPSQMLRTGNNFTFSYTFEDVPFHSSYAHSQSLDRLMNPLIDQYLYYLSRTNTPSGTTTQSRLQFSQAGASDIRDQSRNWLPGPCYRQQRVSKTSADNNNSEYSWTGATKYHLNGRDSLVNPGPAMASHKDDEEKFFPQSGVLIFGKQGSEKTNVDIEKVMITDEEEIRTTNPVATEQYGSVSTNLQRGNLAKADTTKNARQAATADVNTQGVLPGMVWQDRDVYLQGPIWAKIPHTDGHFHPSPLMGGFGLKHPPPQILIKNTPVPANPSTTFSAAKFASFITQYSTGQVSVEIEWELQKENSKRWNPEIQYTSNYNKSVNVDFTVDTNGVYSEPRPIGTRYLTRNL

SEQ ID NO: 26 - protein, 745 aa, Artificial Sequence
  Amino acid sequence of AAV2 seq5 capsid (708V)
MAADGYLPDWLEDTLSEGIRQWWKLKPGPPPPKPAERHKDDSRGLVLPGYKYLGPFNGLDKGEPVNEADAAALEHDKAYDRQLDSGDNPYLKYNHADAEFQERLKEDTSFGGNLGRAVFQAKKRVLEPLGLVEEPVKTAPGKKRPVEHSPVEPDSSSGTGKAGQQPARKRLNFGQTGDADSVPDPQPLGQPPAAPSGLGTNTMATGSGAPMADNNEGADGVGNSSGNWHCDSTWMGDRVITTSTRTWALPTYNNHLYKQISSQSGASNDNHYFGYSTPWGYFDFNRFHCHFSPRDWQRLINNNWGFRPKRLNFKLFNIQVKEVTQNDGTTTIANNLTSTVQVFTDSEYQLPYVLGSAHQGCLPPFPADVFMVPQYGYLTLNNGSQAVGRSSFYCLEYFPSQMLRTGNNFTFSYTFEDVPFHSSYAHSQSLDRLMNPLIDQYLYYLSRTNTPSGTTTQSRLQFSQAGASDIRDQSRNWLPGPCYRQQRVSKTSADNNNSEYSWTGATKYHLNGRDSLVNPGPAMASHKDDEEKFFPQSGVLIFGKQGSEKTNVDIEKVMITDEEEIRTTNPVATEQYGSVSTNLQRGNLAKDDTTRNARQAATADVNTQGVLPGMVWQDRDVYLQGPIWAKIPHTDGHFHPSPLMGGFGLKHPPPQILIKNTPVPANPSTTFSAAKFASFITQYSTGQVSVEIEWELQKENSKRWNPEIQYTSNYNKSVNVDFTVDTNGVYSEPRPIGTRYLTRNL

SEQ ID NO: 27 - protein, 745 aa, Artificial Sequence
  Amino acid sequence of AAV2 seq6 capsid (708V)
MAADGYLPDWLEDTLSEGIRQWWKLKPGPPPPKPAERHKDDSRGLVLPGYKYLGPFNGLDKGEPVNEADAAALEHDKAYDRQLDSGDNPYLKYNHADAEFQERLKEDTSFGGNLGRAVFQAKKRVLEPLGLVEEPVKTAPGKKRPVEHSPVEPDSSSGTGKAGQQPARKRLNFGQTGDADSVPDPQPLGQPPAAPSGLGTNTMATGSGAPMADNNEGADGVGNSSGNWHCDSTWMGDRVITTSTRTWALPTYNNHLYKQISSQSGASNDNHYFGYSTPWGYFDFNRFHCHFSPRDWQRLINNNWGFRPKRLNFKLFNIQVKEVTQNDGTTTIANNLTSTVQVFTDSEYQLPYVLGSAHQGCLPPFPADVFMVPQYGYLTLNNGSQAVGRSSFYCLEYFPSQMLRTGNNFTFSYTFEDVPFHSSYAHSQSLDRLMNPLIDQYLYYLSRTNTPSGTTTQSRLQFSQAGASDIRDQSRNWLPGPCYRQQRVSKTSADNNNSEYSWTGATKYHLNGRDSLVNPGPAMASHKDDEEKFFPQSGVLIFGKQGSEKTNVDIEKVMITDEEEIRTTNPVATEQYGSVSTNLQRGNLALADTTKNARQAATADVNTQGVLPGMVWQDRDVYLQGPIWAKIPHTDGHFHPSPLMGGFGLKHPPPQILIKNTPVPANPSTTFSAAKFASFITQYSTGQVSVEIEWELQKENSKRWNPEIQYTSNYNKSVNVDFTVDTNGVYSEPRPIGTRYLTRNL

SEQ ID NO: 28 - protein, 304 aa, Artificial Sequence
  Sequence of CMV enhancer
CGTTACATAACTTACGGTAAATGGCCCGCCTGGCTGACCGCCCAACGACCCCCGCCCATTGACGTCAATAATGACGTATGTTCCCATAGTAACGCCAATAGGGACTTTCCATTGACGTCAATGGGTGGAGTATTTACGGTAAACTGCCCACTTGGCAGTACATCAAGTGTATCATATGCCAAGTACGCCCCCTATTGACGTCAATGACGGTAAATGGCCCGCCTGGCATTATGCCCAGTACATGACCTTATGGGACTTTCCTACTTGGCAGTACATCTACGTATTAGTCATCGCTATTACCATG

SEQ ID NO: 29 - protein, 309 aa, Artificial Sequence
  Sequence of CMV promoter
TGCTGATGCGGTTTTGGCAGTACACCAATGGGCGTGGATAGCGGTTTGACTCACGGGGATTTCCAAGTCTCCACCCCATTGACGTCAATGGGAGTTTGTTTTGGCACCAAAATCAACGGGACTTTCCAAAATGTCGTAATAACCCCGCCCCGTTGACGCAAATGGGCGGTAGGCGTGTACGGTGGGAGGTCTATATAAGCAGAGCTCGTTTAGTGAACCGTCAGATCGCCTGGAGAGGCCATCCACGCTGTTTTGACCTCCATAGTGGACACCGGGACCGATCCAGCCTCCGCGTCTCAGGGGAAGCTT

SEQ ID NO: 30 - protein, 43 aa, Artificial Sequence
  Sequence of 5'UTR
CTTGTTCTTTTTGCAGAAGCTCAGAATAAACGCTCAACTTTGG

SEQ ID NO: 31 - protein, 6 aa, Artificial Sequence
  Kozak Sequence
GCCACC

SEQ ID NO: 32 - protein, 133 aa, Artificial Sequence
  Sequence of 3'UTR
GTCTAGAAACCAGCCTCAAGAACACCCGAATGGAGTCTCTAAGCTACATAATACCAACTTACACTTTACAAAATGTTGTCCCCCAAAATGTAGCCATTCGTATCTGCTCCTAATAAAAAGAAAGTTTCTTCAC

SEQ ID NO: 33 - protein, 589 aa, Artificial Sequence
  Sequence of WPRE
AATCAACCTCTGGATTACAAAATTTGTGAAAGATTGACTGGTATTCTTAACTATGTTGCTCCTTTTACGCTATGTGGATACGCTGCTTTAATGCCTTTGTATCATGCTATTGCTTCCCGTATGGCTTTCATTTTCTCCTCCTTGTATAAATCCTGGTTGCTGTCTCTTTATGAGGAGTTGTGGCCCGTTGTCAGGCAACGTGGCGTGGTGTGCACTGTGTTTGCTGACGCAACCCCCACTGGTTGGGGCATTGCCACCACCTGTCAGCTCCTTTCCGGGACTTTCGCTTTCCCCCTCCCTATTGCCACGGCGGAACTCATCGCCGCCTGCCTTGCCCGCTGCTGGACAGGGGCTCGGCTGTTGGGCACTGACAATTCCGTGGTGTTGTCGGGGAAATCATCGTCCTTTCCTTGGCTGCTCGCCTGTGTTGCCACCTGGATTCTGCGCGGGACGTCCTTCTGCTACGTCCCTTCGGCCCTCAATCCAGCGGACCTTCCTTCCCGCGGCCTGCTGCCGGCTCTGCGGCCTCTTCCGCGTCTTCGCCTTCGCCCTCAGACGAGTCGGATCTCCCTTTGGGCCGCCTCCCCGC

SEQ ID NO: 34 - protein, 140 aa, Artificial Sequence
  Sequence of SV40polyA
CCTAGGTAAGATACATTGATGAGTTTGGACAAACCACAACTAGAATGCAGTGAAAAAAATGCTTTATTTGTGAAATTTGTGATGCTATTGCTTTATTTGTAACCATTATAAGCTGCAATAAACAAGTTATCGATAGATCT

SEQ ID NO: 35 - protein, 7 aa, Artificial Sequence
  Variant AAV2 capsid protein
  VARIANT (1)..(1): Xaa can be L or K
  VARIANT (2)..(2): Xaa can be G, D or A
  VARIANT (3)..(3): Xaa can be D or E
  VARIANT (6)..(6): Xaa can be R or K
  VARIANT (7)..(7): Xaa can be P or N
XXXTTXX

SEQ ID NO: 36 - protein, 11 aa, Artificial Sequence
  Variant AAV2 capsid protein
  VARIANT (1)..(1): Xaa can be deleted, or can be A, L, G, S or T
  VARIANT (2)..(2): Xaa can be deleted, or can be A, L, G, S or T
  VARIANT (3)..(3): Xaa can be L or K
  VARIANT (4)..(4): Xaa can be G, D or A
  VARIANT (5)..(5): Xaa can be D or E
  VARIANT (8)..(8): Xaa can be R or K
  VARIANT (9)..(9): Xaa can be P or N
  VARIANT (10)..(10): Xaa can be deleted, or can be A, L, G, S or T
  VARIANT (11)..(11): Xaa can be deleted, or can be A, L, G, S or T
XXXXXTTXXXX

SEQ ID NO: 37 - protein, 736 aa, Artificial Sequence
  Amino acid sequence of AAV9 capsid
MAADGYLPDWLEDNLSEGIREWWALKPGAPQPKANQQHQDNARGLVLPGYKYLGPGNGLDKGEPVNAADAAALEHDKAYDQQLKAGDNPYLKYNHADAEFQERLKEDTSFGGNLGRAVFQAKKRLLEPLGLVEEAAKTAPGKKRPVEQSPQEPDSSAGIGKSGAQPAKKRLNFGQTGDTESVPDPQPIGEPPAAPSGVGSLTMASGGGAPVADNNEGADGVGSSSGNWHCDSQWLGDRVITTSTRTWALPTYNNHLYKQISNSTSGGSSNDNAYFGYSTPWGYFDFNRFHCHFSPRDWQRLINNNWGFRPKRLNFKLFNIQVKEVTDNNGVKTIANNLTSTVQVFTDSDYQLPYVLGSAHEGCLPPFPADVFMIPQYGYLTLNDGSQAVGRSSFYCLEYFPSQMLRTGNNFQFSYEFENVPFHSSYAHSQSLDRLMNPLIDQYLYYLSKTINGSGQNQQTLKFSVAGPSNMAVQGRNYIPGPSYRQQRVSTTVTQNNNSEFAWPGASSWALNGRNSLMNPGPAMASHKEGEDRFFPLSGSLIFGKQGTGRDNVDADKVMITNEEEIKTTNPVATESYGQVATNHQSAQAQAQTGWVQNQGILPGMVWQDRDVYLQGPIWAKIPHTDGNFHPSPLMGGFGMKHPPPQILIKNTPVPADPPTAFNKDKLNSFITQYSTGQVSVEIEWELQKENSKRWNPEIQYTSNYYKSNNVEFAVNTEGVYSEPRPIGTRYLTRNL

SEQ ID NO: 38 - protein, 448 aa, Artificial Sequence
  Sequence of aflibercept protein
MPLLLLLPLLWAGALASDTGRPFVEMYSEIPEIIHMTEGRELVIPCRVTSPNITVTLKKFPLDTLIPDGKRIIWDSRKGFIISNATYKEIGLLTCEATVNGHLYKTNYLTHRQTNTIIDVVLSPSHGIELSVGEKLVLNCTARTELNVGIDFNWEYPSSKHQHKKLVNRDLKTQSGSEMKKFLSTLTIDGVTRSDQGLYTCAASSGLMTKKNSTFVRVHEKDKTHTCPPCPAPELLGGPSVFLFPPKPKDTLMISRTPEVTCVVVDVSHEDPEVKFNWYVDGVEVHNAKTKPREEQYNSTYRVVSVLTVLHQDWLNGKEYKCKVSNKALPAPIEKTISKAKGQPREPQVYTLPPSRDELTKNQVSLTCLVKGFYPSDIAVEWESNGQPENNYKTTPPVLDSDGSFFLYSKLTVDKSRWQQGNVFSCSVMHEALHNHYTQKSLSLSPGK

SEQ ID NO: 39 - DNA, 1347 bp, Artificial Sequence
  Nucleic acid sequence 1 of aflibercept
atgcccctgctcctgctcctgcccctgctgtgggccggcgccctggctagcgacaccggcagacccttcgtggagatgtacagcgagatccccgagatcatccacatgaccgagggcagagagctggtgatcccctgcagagtgacaagccccaacatcaccgtgaccctgaaaaaattccctctggacaccctgatccccgacggcaagagaatcatctgggacagcagaaagggcttcatcatcagcaacgccacctacaaggagatcggcctgctgacctgcgaggccaccgtgaacggccacctgtacaagaccaactacctgacccacagacagaccaacaccatcatcgacgtggtgctgagccctagccacggcatcgagctgagcgtgggcgagaagctggtgctgaactgcaccgctagaaccgagctgaacgtgggcatcgacttcaactgggagtaccctagcagcaagcatcagcacaagaagctggtgaacagagacctgaagacacagagcggcagcgagatgaagaagttcctgagcaccctgaccatcgacggcgtgacaagaagcgaccaaggcctgtacacctgcgccgctagcagcggcctgatgaccaagaagaacagcaccttcgtgagagtgcatgagaaggacaagacccacacctgccccccctgccccgctcctgaactgctgggcggccctagcgtgttcctgttcccccccaagcccaaggacacactcatgatcagcagaacccccgaggtgacctgcgtggtcgtggacgtgagccacgaggaccccgaggtgaagttcaactggtacgtggacggcgtggaggtgcacaacgccaagaccaagcctagagaggagcagtacaacagcacctacagagtggtgagcgtgctgaccgtgctgcaccaagactggctgaacggcaaggagtacaagtgcaaggtgagcaacaaggccctgcccgcccccatcgagaagaccatcagcaaggccaaggggcagcctagagagccccaagtgtacaccctgccccctagcagagacgagctgaccaagaaccaagtgagcctgacctgcctggtgaagggcttctaccctagcgacatcgccgtggagtgggagagcaacgggcagcccgagaacaactacaagaccaccccccccgtgctggacagcgacggcagcttcttcctgtacagcaagctgaccgtggacaagagcagatggcagcaaggcaacgtgttcagctgcagcgtgatgcacgaggccctgcacaaccactacacacagaagagcctgagcctgagccccggcaagtga

SEQ ID NO: 40 - DNA, 1347 bp, Artificial Sequence
  Nucleic acid sequence 2 of aflibercept
atgcctctgctcctgctgctccctctgctgtgggccggcgccctggccagcgacacaggccgccccttcgtggaaatgtacagcgagatccctgagatcatccacatgacagagggccgggaactggtcatcccttgtagagtgacatctccaaacatcaccgtgaccctgaaaaagttccccctggacacactgatccctgacggcaaaagaatcatctgggattcccggaagggcttcatcatcagcaatgccacctacaaggaaatcggactgctgacctgtgaagccacagtgaacggccacctgtacaagaccaactacctgacccataggcagaccaataccatcatcgatgtggtgctgtctccttctcacggcatcgagctcagcgtcggcgagaaactggtgctgaactgcaccgccagaaccgagctgaacgtgggcatcgacttcaactgggaataccccagttctaagcaccagcacaagaaactggttaatagagatctgaagacccaaagcggcagcgagatgaaaaagtttctgtctacactgacaattgacggtgttaccagaagcgatcagggcctgtatacatgcgccgcttctagcggcctgatgaccaagaagaacagcaccttcgtgcgggtgcacgagaaggacaagacccacacctgccccccctgtccagctcctgaactgctgggaggccctagcgtgttcctgttccctccaaagcctaaggacacccttatgattagcagaacacctgaggtgacctgcgtggtggtcgacgtgtcccacgaggaccccgaggtgaaatttaactggtacgtggatggcgtggaagttcacaacgccaagaccaagcccagagaggaacagtacaacagcacatatagagtggtgtccgtgctgaccgttctgcaccaggactggctgaatggaaaagagtacaagtgcaaggtgtccaacaaggccctgcctgcccctatcgagaagactatcagcaaggctaagggccaacctcgggaaccccaggtgtacaccctgccccccagccgggacgagctgacaaagaaccaggtgtccctgacatgcctggtgaagggattttaccctagcgatatcgccgtggaatgggagagcaacggccagcctgagaacaactacaaaacgacccctcctgtgctggactctgatggcagcttcttcctgtacagcaagctgaccgtggacaagagcagatggcagcagggcaacgtgttctcatgcagcgtgatgcacgaggccctgcataatcactacacccagaaaagcctgagcctgagccctggcaagtga

SEQ ID NO: 41 - DNA, 1347 bp, Artificial Sequence
  Nucleic acid sequence 3 of aflibercept
atgccactgctcttgcttttgcccttgctttgggctggtgcccttgcctcagacactggaaggccgttcgtagaaatgtactccgagatccctgaaataatccacatgacggaggggcgagagttggtgataccatgtcgagttacgagcccgaatattacagtaacattgaagaaattcccactcgacactctcattccagatggtaagagaattatatgggattcacgaaagggcttcattatatctaacgctacttacaaagagataggcttgctcacatgcgaggcaactgtcaatggccacttgtataaaaccaattatctcacacataggcagactaatacgataatagacgttgtcctttctccgagccatggcattgaattgagtgtcggtgagaagctcgtattgaactgcactgctaggaccgagcttaacgtagggatcgactttaactgggagtacccatcatcaaagcatcagcataaaaagctcgtcaaccgggaccttaagacgcagagtggctcagagatgaagaagttcctttctacactgaccatcgatggtgtaaccagaagtgaccagggactctatacctgtgccgcatcctccggccttatgacgaagaaaaacagcacatttgttcgggtccacgagaaggacaagactcatacgtgtccgccgtgtccagccccagaattgctcggggggccttccgtgtttctgttccctccaaagccaaaggacacgcttatgatttcaaggactcccgaagtcacctgcgtcgtggttgacgtttctcatgaggacccagaggtgaaattcaactggtacgtggatggagtagaggtacataacgccaaaacaaaaccacgagaagagcagtataactcaacgtatcgggtagtttctgtgcttacggttctccaccaagattggttgaatggaaaagagtataagtgtaaagtctcaaacaaagccctgccggcacccatcgagaagaccattagcaaagcaaaaggccaacctagagaaccgcaggtgtacacgttgccaccgtcaagggatgaacttacgaagaatcaagtatcactcacatgtttggttaaaggattttatcccagcgacatcgccgtagaatgggagagtaacggccagcctgaaaataactataagacgacaccccctgttttggattctgacggttcattttttttgtatagtaaactcacagtcgacaagagtcgctggcaacaaggtaatgtatttagctgtagcgtgatgcatgaagctttgcacaaccactatacacagaagtccttgtctctgtctccgggaaaatga